European Patent Specification EP 3 753 922 B1, published March 26, 2025. Title: Composition for detecting dsRNA comprising merocyanine, salts thereof, or isomer thereof and Method for providing information on diagnosing cancer using analyzing dsRNA expression. Applicant: KAIST. The sequence listing filed with the application follows.

SEQUENCE LISTING (30 sequences)

SEQ ID NO: 1 - DNA, 19 bp, Artificial Sequence
  Primer sequence for qPCR
tgattttgcaggctcacag

SEQ ID NO: 2 - DNA, 20 bp, Artificial Sequence
  Primer sequence for qPCR
tcctcccaaatctcatgtcc

SEQ ID NO: 3 - DNA, 19 bp, Artificial Sequence
  Primer sequence for qPCR
ctgctccccacagtgtctc

SEQ ID NO: 4 - DNA, 19 bp, Artificial Sequence
  Primer sequence for qPCR
caggttcaaactgttccag

SEQ ID NO: 5 - DNA, 20 bp, Artificial Sequence
  Primer sequence for qPCR
ggagcttcctgattggcaga

SEQ ID NO: 6 - DNA, 20 bp, Artificial Sequence
  Primer sequence for qPCR
atgtagggtggcaagcactg

SEQ ID NO: 7 - DNA, 20 bp, Artificial Sequence
  Primer sequence for qPCR
tattgccgtactgtgggctg

SEQ ID NO: 8 - DNA, 20 bp, Artificial Sequence
  Primer sequence for qPCR
tggaacagagcccttccttg

SEQ ID NO: 9 - DNA, 20 bp, Artificial Sequence
  Primer sequence for qPCR
aaggtgtagcccatgaggtg

SEQ ID NO: 10 - DNA, 20 bp, Artificial Sequence
  Primer sequence for qPCR
ggccctgttcaactaagcac

SEQ ID NO: 11 - DNA, 21 bp, Artificial Sequence
  Primer sequence for qPCR
tcaaactcaaactacgccctg

SEQ ID NO: 12 - DNA, 21 bp, Artificial Sequence
  Primer sequence for qPCR
gttgtgataagggtggagagg

SEQ ID NO: 13 - DNA, 19 bp, Artificial Sequence
  Primer sequence for qPCR
ctaggccttcttacgagcc

SEQ ID NO: 14 - DNA, 20 bp, Artificial Sequence
  Primer sequence for qPCR
tttgggttgaggtgatgatg

SEQ ID NO: 15 - DNA, 21 bp, Artificial Sequence
  Primer sequence for qPCR
tcaaactcaaactacgccctg

SEQ ID NO: 16 - DNA, 21 bp, Artificial Sequence
  Primer sequence for qPCR
gctgtgataagggtggagagg

SEQ ID NO: 17 - DNA, 21 bp, Artificial Sequence
  Primer sequence for qPCR
ctcacactcattctcaacccc

SEQ ID NO: 18 - DNA, 20 bp, Artificial Sequence
  Primer sequence for qPCR
tgtttgtcgtaggcagatgg

SEQ ID NO: 19 - DNA, 20 bp, Artificial Sequence
  Primer sequence for qPCR
ctaggccttcttacgagcca

SEQ ID NO: 20 - DNA, 20 bp, Artificial Sequence
  Primer sequence for qPCR
tttgggttgaggtgatgatg

SEQ ID NO: 21 - DNA, 21 bp, Artificial Sequence
  Primer sequence for qPCR
tgctgtgggtgaaagagtagt

SEQ ID NO: 22 - DNA, 20 bp, Artificial Sequence
  Primer sequence for qPCR
cccataatcataaaagcccc

SEQ ID NO: 23 - DNA, 22 bp, Artificial Sequence
  Primer sequence for qPCR
caattataccctagccaacccc

SEQ ID NO: 24 - DNA, 22 bp, Artificial Sequence
  Primer sequence for qPCR
ggatagtaatagggcaaggacg

SEQ ID NO: 25 - DNA, 21 bp, Artificial Sequence
  Primer sequence for qPCR
gccataacccaataccaaacg

SEQ ID NO: 26 - DNA, 20 bp, Artificial Sequence
  Primer sequence for qPCR
ttgaggttgcggtctgttag

SEQ ID NO: 27 - DNA, 22 bp, Artificial Sequence
  Primer sequence for qPCR
ctagtcctgtatgcccttttcc

SEQ ID NO: 28 - DNA, 21 bp, Artificial Sequence
  Primer sequence for qPCR
gtaaaggatgcgtagggatgg

SEQ ID NO: 29 - DNA, 21 bp, Artificial Sequence
  Primer sequence for qPCR
ccttttaccactccagcctag

SEQ ID NO: 30 - DNA, 21 bp, Artificial Sequence
  Primer sequence for qPCR
ctcctgatgcgagtaatacgg